European Patent Application EP 4 512 413 A1, published February 26, 2025. Title: IL-27蛋白在制备治疗和/或延缓阿尔茨海默症的产品的应用. Applicant: 广东暨安特博生物科技有限公司. The sequence listing filed with the application follows.

SEQUENCE LISTING (2 sequences)

SEQ ID NO: 1 - protein, 234 aa, synthetic construct
MGQVTGDLGWRLSLLLLPLLLVQAGSWGFPTDPLSLQELRREFTVSLYLARKLLSEVQGYVHSFAESRLPGVNLDLLPLGYHLPNVSLTFQAWHHLSDSERLCFLATTLRPFPAMLGGLGTQGTWTSSEREQLWAMRLDLRDLHRHLRFQVLAAGFKCSKEEEDKEEEEEEEEEEKKLPLGALGGPNQVSSQVSWPQLLYTYQLLHSLELVLSRAVRDLLLLSLPRRPGSAWDS

SEQ ID NO: 2 - DNA, 6017 bp, synthetic construct
  source 1..6017: mol_type = other DNA
cttagtgaacacaaagctgaaagtacaagtaggacagaaagtgaaactgggcgcagcccccagtataagacccccctacccaggagatggctgcacacagaggctgggccctgacatgggccaggtgacaggagaccttggctggcgtgagttggaagcggcgactgggctgagggctgggaggtttggtggagcccaggagaggttgggaaagtttgacaggtagggttggggcagaaagttgaggggcaacacgttggccacgtagacaggcatggctagctgaccacgggaatgagactagtgtaagtgggcaggggttagagcagtggaattatggttggctgggtaagtgatagcagtgtctgggatgtgtcaggaggactggacaggcaacctggccaggagcaggactaaacagacaaatgaagagtgtagagggaagaggctgagaaccgaggacagtcagaggaacggcacaggggagctggtaagagcggtgactgggaccaagggggcaacctctctgggtaaaggtctctaacttacccaaggtctggaacttagaaggttgcccagtctgcagctgggagctgaaggactcggaacagagttgtaggaagaggggcaagttgtaggctgggtaggctcaagggctggagcatgagggcgggattctctacaaaggggtcttggggtgtctagaattttgagaggtggtaagtgggtatgagctggcacaccttagtctgggatgtaatatttaccaaggcctaagggttcatgccttctccccatcctagagctaggaagaattctatttagtctccaggatattagggagtcagaatggttctcaagccaagaaacctgaatgccagagatctcaatcactgcccacttctgaaagtacatggggaaaatagatgtcgtcccccacgcccccaagctttcattaactactgctgagggcactttagggaggtttatagattatgaatggatagaagggacctggagaggagcaagggtggggagagacttggggatagttttggtttgggtttcggggagaattgtgtaactcccgcttgagagagaaaccactgaagattgccttcttcccagagctcccacttcacagccctgctccctcttactacaaattgcagggcttgaagtcccctgaaaagtcagatagcatgactctcactccacagctgggagcctgggacacaaaaataagaggtgacctgctcaaggcaggatgaagacactagcctccccctccatcagtgccatccccaccacatgtcccttccaggaccatactgctaatttaccctagaagggctcagtgcacagtggcatattttccatatgagtccctagaatagaaccactggctttgccaggtcttccctagggccctaggtctgtttaaagcctcagggctgtctgggtgaacccaaggaatccttggcagaacacagtgttgccacctctggagcaggtgggttcttcctctgagttccctggggatagagtactggcctgtgtttgggtggatctggagtccaaccctgcctccctgacctctcactgactaaccgtggctagtcactttacccagtctcaagggctagggcacacacatgcagttatgtaggctgggcactggaaaaggcaattgactaagggatctagttggagtgtgtgtattaagatcctgcttttggggcttggaggtggtagcacacacctttaatcccagcacttgggaggcagaggcaggcagatttctgagtacaaggccagcctggtctacagagtgagttccaggacagccatggctacacagagaaaccctgtctagaaaacaaaacgaaacaacaacaacaacaacaaagatcctgcctttggtgttcttacaacagtgtgcagagtgacatgggggtagcctctgtggtccaaatgatggttctaagagggtagcttgaagatgccaaagagactcagtgcttgtatagatcggtttcttccttctccagggttctccagcctttatcttgtcacctttcctcctttctccagggctcagcctgttgctgctacccttgcttctggtacaagctggttcctgggggttcccaacagaccccctgagccttcaagagctgcgcagggaattcacagtcagcctgtaccttgccaggaagctgctctctgaggttcagggctatgtccacagctttgtgagtctccttagcgcaattgggtctggaggtgaggacacccccaagtcccactggccctcactaacagaatttaaccctcaggctgaatctcgattgccaggagtgaacctggacctcctgcccctgggataccatcttcccaatgtttccctgactttccaggcatggcatcacctctctgtaagtgaacggcaaggggatggggagactggcagtaaagtatggtacatagacaagtgtttgagcagatgtggatctgcaggtttgtatggctaatatgtctctgtatgtaaaggtgaagctggaagctgagggtagtggtacacatctgtaatcccaatacttgggaggcagagactaggatttgaggaagatagaggaacaaaggagagggagctgggatttgaaagtggggaccgcaagatggtgagcatgacactgggggaagaggtgggactgggaatggaggtagctatgggaaagagatgggctgacgactgtgatgggagtggggtcaagtcagagagaagacagctgtggatatgggtgaaaattgggttggagatgaaagaaggaagttcaatgggcacgctgaatttgagcctgtggagcgaggtggatttgggttaagaataagaatgagggctggagagatggctcagcggttaagggcactgactgctctgccagaggcagtgagttcaattcccagctggtggctcacaaccatctgtgatgggatccagtgcatgaatgggaatgaggcgggaaagctggtggctcacaaccatctgtgatgggatccagtgcatgaatgggaatgaggcgggaaagctggtggagatgccagcacaagatgtgactgacaggttgtatggatggcaacggaagggacagaatgaagctgtgggtggagggagtgggttgaggagatgagtatggggccaaggagacaggactgacctcacaatgatagaagaaggcaagaataaatccaaggagcctagtgatatggctcaggagagaaaggctcttgctgccaaagctaacaacctgagttaaatccctggagcccacacggtaggagagaaccaatttcaggaagtcgtcctctgatgttcatagacatgtgcacaggtacacacatacacatgctataaatagatgtgacataatactttttgttgttgttttggctctttgagacaagcatcactatttgccctggctgttctggaactccctaagtagaccaggctgacctctgactcacagaggtcctcctatatctgcctgctgagtgctgggattagatgtgtgtgctgccatgcatgaggtaataaaaaatttagctggtagtggtggcacacaccggtaggatttgctgaaggaggcagaggcaggaggatcacgagttcgaggccagcctaggctacagagtgagttccaggacagccagggctacacagagaaaccctgtctcaaaaaaaaaaaaaaaaaaaaaaaaaaaaaaaaaaatttaaagtgtaaacttgtgaatgaaatggaagctagaataaaaaagagacccatataaagatggcactcaatttggtgtttttccccttctcttcaataggactctgagagactctgcttcctcgctaccacacttcggcccttccctgccatgctgggagggctggggacccaggggacctggaccagctcagagagggagcagctgtgggccatgaggctggatctccgggacctgcacaggcacctccgctttcaggtagagtgcgcactgtacccttgaccccggggatctacaagcaaactggactcactggctctcttttgaaacacctcccagaatcaggttgaagaagcctagtgagacacttcagcttctgtgagtgagtagcggccctagagcctggctctgcccaaagtctctgcctgctcttgagggctggactccagtgaaagaatagccatgggacaccagggcagcccctgtcgtcatcgggcccagtatccgtcccttctccctccagttccgacttcactcggattctccgaggcgggtcaaagggcaatagaaattttaccttagtaaaaagaaaattgaaaatgcaaaacaggaactacctgtgtcaccccctctgatcctgaaaaatccttaacagcagagaatttcctgaccagtgatccccagagcaaagcagtcccacccagtttggagcatcttgctctaccacgaccatttttaaaaatagatagacagacagacagacagacaggtaagggggctggagagaaagtcccgtcgtttacagcactggctgctcttcccgaggacttgggtccaatccccagcaactcaaccatttcacaaccatctgtaactccagttctagggtatctgacgccttttctctgctccttggcacttggtaagtggtgcacatacacacaggcagaacactcatacacataaaataaatttaatagttttttttttttaaatctagtacgccaagtgtggtgatgcattcctgtcgtctcaaacacttggttggttgaggcaggagaattgtgatttcaaggccacactgtaactatagaggaagattctgtaaaataaacaaacacaagaaacagagctggagagatggcaagagcagcacttgctggtcttgcagaggataaatgctaacacccagcactctctctggccttgaagaacaccagtcatacaggcagtgcacatacatacatgcagacaaagggctcgtatatacgaaataaaaaaataaatcatatatatatatgacagctcagcagtcaagaacacagtttgtcttacaaaagacccaagtttgagtcccagcatccacatagtgactcacaaccatcctcaaatccagttccaggggacctgatgtctcgtctcacccccttaagcactgcacacatgtggtacacacccatacacattaaataaataaataaataaataataggaatgttaaagggaaaagaaataaaatgcaagatttaaataaagacatgactagattagataaagactttgaccctgtaagtctgagggagaggctaccagagcaaccagggcctgtggttactgatgtcactggaggtgatgggcagcagaaggaatggagactctctctggttcttgatgtggccctgtgtgtctttcctcataggtgctggctgcaggattcaaatgttcaaaggaggaggaggacaaggaggaagaggaagaggaggaagaagaagaaaagaagctgcccctaggggctctgggtggccccaatcaggtgtcatcccaagtgtcctggccccagctgctctatacctaccagctccttcactccctggagcttgtcctgtctcgggctgttcgggacctgctgctgctgtccctgcccaggcgcccaggctcagcctgggattcctaacacctagcttcaagccctatggagtgaccttccagctccctccctcgcccgttaagactctaaggctggagtctggccaatcacaggacaggctctagctcgtttgccttagaccaggcagggcttcactagctcccagccctgacccaataatttaaaagccctccagtccttaccagatatttatttcttggatatttatttatttttaagaaatggtttatttattgtttcactcttgagttaggccaccatgctgggtgcctaataaagccatccagcccgg